European Patent Specification EP 3 384 926 B1, published October 9, 2024. Title: CANCER VACCINE COMPOSITION. Applicant: International Institute of Cancer Immunology, Inc. The sequence listing filed with the application follows.

SEQUENCE LISTING (75 sequences)

SEQ ID NO: 1 - protein, 449 aa, Human
MGSDVRDLNALLPAVPSLGGGGGCALPVSGAAQWAPVLDFAPPGASAYGSLGGPAPPPAPPPPPPPPPHSFIKQEPSWGGAEPHEEQCLSAFTVHFSGQFTGTAGACRYGPFGPPPPSQASSGQARMFPNAPYLPSCLESQPAIRNQGYSTVTFDGTPSYGHTPSHHAAQFPNHSFKHEDPMGQQGSLGEQQYSVPPPVYGCHTPTDSCTGSQALLLRTPYSSDNLYQMTSQLECMTWNQMNLGATLKGVAAGSSSSVKWTEGQSNHSTGYESDNHTTPILCGAQYRIHTHGVFRGIQDVRRVPGVAPTLVRSASETSEKRPFMCAYPGCNKRYFKLSHLQMHSRKHTGEKPYQCDFKDCERRFSRSDQLKRHQRRHTGVKPFQCKTCQRKFSRSDHLKTHTRTHTGKTSEKPFSCRWPSCQKKFARSDELVRHHNMHQRNMTKLQLAL

SEQ ID NO: 2 - protein, 9 aa, Artificial
  Synthetic peptide
SLGEQQYSV

SEQ ID NO: 3 - protein, 9 aa, Artificial
  Synthetic peptide
RMFPNAPYL

SEQ ID NO: 4 - protein, 9 aa, Artificial
  Synthetic peptide
GLGEQQYSV

SEQ ID NO: 5 - protein, 9 aa, Artificial
  Synthetic peptide
ALGEQQYSV

SEQ ID NO: 6 - protein, 9 aa, Artificial
  Synthetic peptide
VLGEQQYSV

SEQ ID NO: 7 - protein, 9 aa, Artificial
  Synthetic peptide
LLGEQQYSV

SEQ ID NO: 8 - protein, 9 aa, Artificial
  Synthetic peptide
ILGEQQYSV

SEQ ID NO: 9 - protein, 9 aa, Artificial
  Synthetic peptide
MLGEQQYSV

SEQ ID NO: 10 - protein, 9 aa, Artificial
  Synthetic peptide
WLGEQQYSV

SEQ ID NO: 11 - protein, 9 aa, Artificial
  Synthetic peptide
FLGEQQYSV

SEQ ID NO: 12 - protein, 9 aa, Artificial
  Synthetic peptide
YLGEQQYSV

SEQ ID NO: 13 - protein, 9 aa, Artificial
  Synthetic peptide
SVGEQQYSV

SEQ ID NO: 14 - protein, 9 aa, Artificial
  Synthetic peptide
SQGEQQYSV

SEQ ID NO: 15 - protein, 9 aa, Artificial
  Synthetic peptide
SIGEQQYSV

SEQ ID NO: 16 - protein, 9 aa, Artificial
  Synthetic peptide
SMGEQQYSV

SEQ ID NO: 17 - protein, 9 aa, Artificial
  Synthetic peptide
SLLEQQYSV

SEQ ID NO: 18 - protein, 9 aa, Artificial
  Synthetic peptide
SLAEQQYSV

SEQ ID NO: 19 - protein, 9 aa, Artificial
  Synthetic peptide
SLVEQQYSV

SEQ ID NO: 20 - protein, 9 aa, Artificial
  Synthetic peptide
SLMEQQYSV

SEQ ID NO: 21 - protein, 9 aa, Artificial
  Synthetic peptide
SLPEQQYSV

SEQ ID NO: 22 - protein, 9 aa, Artificial
  Synthetic peptide
SLWEQQYSV

SEQ ID NO: 23 - protein, 9 aa, Artificial
  Synthetic peptide
SLFEQQYSV

SEQ ID NO: 24 - protein, 9 aa, Artificial
  Synthetic peptide
SLYEQQYSV

SEQ ID NO: 25 - protein, 9 aa, Artificial
  Synthetic peptide
SLSEQQYSV

SEQ ID NO: 26 - protein, 9 aa, Artificial
  Synthetic peptide
SLIEQQYSV

SEQ ID NO: 27 - protein, 9 aa, Artificial
  Synthetic peptide
GMFPNAPYL

SEQ ID NO: 28 - protein, 9 aa, Artificial
  Synthetic peptide
AMFPNAPYL

SEQ ID NO: 29 - protein, 9 aa, Artificial
  Synthetic peptide
VMFPNAPYL

SEQ ID NO: 30 - protein, 9 aa, Artificial
  Synthetic peptide
LMFPNAPYL

SEQ ID NO: 31 - protein, 9 aa, Artificial
  Synthetic peptide
IMFPNAPYL

SEQ ID NO: 32 - protein, 9 aa, Artificial
  Synthetic peptide
MMFPNAPYL

SEQ ID NO: 33 - protein, 9 aa, Artificial
  Synthetic peptide
WMFPNAPYL

SEQ ID NO: 34 - protein, 9 aa, Artificial
  Synthetic peptide
FMFPNAPYL

SEQ ID NO: 35 - protein, 9 aa, Artificial
  Synthetic peptide
YMFPNAPYL

SEQ ID NO: 36 - protein, 9 aa, Artificial
  Synthetic peptide
RVFPNAPYL

SEQ ID NO: 37 - protein, 9 aa, Artificial
  Synthetic peptide
RQFPNAPYL

SEQ ID NO: 38 - protein, 9 aa, Artificial
  Synthetic peptide
RAFPNAPYL

SEQ ID NO: 39 - protein, 9 aa, Artificial
  Synthetic peptide
RLFPNAPYL

SEQ ID NO: 40 - protein, 9 aa, Artificial
  Synthetic peptide
RIFPNAPYL

SEQ ID NO: 41 - protein, 9 aa, Artificial
  Synthetic peptide
RMIPNAPYL

SEQ ID NO: 42 - protein, 9 aa, Artificial
  Synthetic peptide
RMLPNAPYL

SEQ ID NO: 43 - protein, 9 aa, Artificial
  Synthetic peptide
RMGPNAPYL

SEQ ID NO: 44 - protein, 9 aa, Artificial
  Synthetic peptide
RMAPNAPYL

SEQ ID NO: 45 - protein, 9 aa, Artificial
  Synthetic peptide
RMVPNAPYL

SEQ ID NO: 46 - protein, 9 aa, Artificial
  Synthetic peptide
RMMPNAPYL

SEQ ID NO: 47 - protein, 9 aa, Artificial
  Synthetic peptide
RMPPNAPYL

SEQ ID NO: 48 - protein, 9 aa, Artificial
  Synthetic peptide
RMWPNAPYL

SEQ ID NO: 49 - protein, 9 aa, Artificial
  Synthetic peptide
RMFPNAPYV

SEQ ID NO: 50 - protein, 9 aa, Artificial
  Synthetic peptide
RMFPNAPYA

SEQ ID NO: 51 - protein, 9 aa, Artificial
  Synthetic peptide
RMFPNAPYI

SEQ ID NO: 52 - protein, 9 aa, Artificial
  Synthetic peptide
RMFPNAPYM

SEQ ID NO: 53 - protein, 9 aa, Artificial
  Synthetic peptide
SLGEQQYSL

SEQ ID NO: 54 - protein, 9 aa, Artificial
  Synthetic peptide
DLGEQQYSV

SEQ ID NO: 55 - protein, 9 aa, Artificial
  Synthetic peptide
ELGEQQYSV

SEQ ID NO: 56 - protein, 9 aa, Artificial
  Synthetic peptide
HLGEQQYSV

SEQ ID NO: 57 - protein, 9 aa, Artificial
  Synthetic peptide
KLGEQQYSV

SEQ ID NO: 58 - protein, 9 aa, Artificial
  Synthetic peptide
NLGEQQYSV

SEQ ID NO: 59 - protein, 9 aa, Artificial
  Synthetic peptide
PLGEQQYSV

SEQ ID NO: 60 - protein, 9 aa, Artificial
  Synthetic peptide
QLGEQQYSV

SEQ ID NO: 61 - protein, 9 aa, Artificial
  Synthetic peptide
RLGEQQYSV

SEQ ID NO: 62 - protein, 9 aa, Artificial
  Synthetic peptide
TLGEQQYSV

SEQ ID NO: 63 - protein, 9 aa, Artificial
  Synthetic peptide
DMFPNAPYL

SEQ ID NO: 64 - protein, 9 aa, Artificial
  Synthetic peptide
EMFPNAPYL

SEQ ID NO: 65 - protein, 9 aa, Artificial
  Synthetic peptide
HMFPNAPYL

SEQ ID NO: 66 - protein, 9 aa, Artificial
  Synthetic peptide
KMFPNAPYL

SEQ ID NO: 67 - protein, 9 aa, Artificial
  Synthetic peptide
NMFPNAPYL

SEQ ID NO: 68 - protein, 9 aa, Artificial
  Synthetic peptide
PMFPNAPYL

SEQ ID NO: 69 - protein, 9 aa, Artificial
  Synthetic peptide
QMFPNAPYL

SEQ ID NO: 70 - protein, 9 aa, Artificial
  Synthetic peptide
SMFPNAPYL

SEQ ID NO: 71 - protein, 9 aa, Artificial
  Synthetic peptide
TMFPNAPYL

SEQ ID NO: 72 - protein, 9 aa, Artificial
  Synthetic peptide
RIFPNAPYI

SEQ ID NO: 73 - protein, 9 aa, Artificial
  Synthetic peptide
RIFPNAPYV

SEQ ID NO: 74 - protein, 9 aa, Artificial
  Synthetic peptide
RLFPNAPYI

SEQ ID NO: 75 - protein, 9 aa, Artificial
  Synthetic peptide
RLFPNAPYV